European Patent Specification EP 4 059 510 B1, published May 21, 2025. Title: ENGINEERED EXTRACELLULAR VESICLES AND USES THEREOF. Applicant: CODIAK BIOSCIENCES. Application PCT/US2018/061679. The sequence listing filed with the application follows.

SEQUENCE LISTING (425 sequences)

SEQ ID NO: 1 - protein, 332 aa, Artificial Sequence
  MARCKS protein
MGAQFSKTAAKGEAAAERPGEAAVASSPSKANGQENGHVKVNGDASPAAAESGAKEELQANGSAPAADKEEPAAAGSGAASPSAAEKGEPAAAAAPEAGASPVEKEAPAEGEAAEPGSPTAAEGEAASAASSTSSPKAEDGATPSPSNETPKKKKKRFSFKKSFKLSGFSFKKNKKEAGEGGEAEAPAAEGGKDEAAGGAAAAAAEAGAASGEQAAAPGEEAAAGEEGAAGGDPQEAKPQEAAVAPEKPPASDETKAAEEPSKVEEKKAEEAGASAAACEAPSAAGPGAPPEQEAAPAEEPAAAAASSACAAPSQEAQPECSPEAPPAEAAE

SEQ ID NO: 2 - protein, 195 aa, Artificial Sequence
  MARCKSL1 protein
MGSQSSKAPRGDVTAEEAAGASPAKANGQENGHVKSNGDLSPKGEGESPPVNGTDEAAGATGDAIEPAPPSQGAEAKGEVPPKETPKKKKKFSFKKPFKLSGLSFKRNRKEGGGDSSASSPTEEEQEQGEIGACSDEGTAQEGKAAATPESQEPQAKGAEASAASEEEAGPQATEPSTPSGPESGPTPASAEQNE

SEQ ID NO: 3 - protein, 227 aa, Artificial Sequence
  BASP1 protein
MGGKLSKKKKGYNVNDEKAKEKDKKAEGAATEEEGTPKESEPQAAAEPAEAKEGKEKPDQDAEGKAEEKEGEKDAAAAKEEAPKAEPEKTEGAAEAKAEPPKAPEQEQAAPGPAAGGEAPKAAEAAAAPAESAAPAAGEEPSKEEGEPKKTEAPAAPAAQETKSDGAPASDSKPGSSEAAPSSKETPAATEAPSSTPKAQGPAASAEEPKPVEAPAANSDQTVTVKE

SEQ ID NO: 4 - protein, 30 aa, Artificial Sequence
  BASP1 fragment
MGGKLSKKKKGYNVNDEKAKEKDKKAEGAA

SEQ ID NO: 5 - protein, 27 aa, Artificial Sequence
  fusion protein
MGGKLSKKKKGYNVNDEKAKEKDKKAE

SEQ ID NO: 6 - protein, 24 aa, Artificial Sequence
  fusion protein
MGGKLSKKKKGYNVNDEKAKEKDK

SEQ ID NO: 7 - protein, 21 aa, Artificial Sequence
  fusion protein
MGGKLSKKKKGYNVNDEKAKE

SEQ ID NO: 8 - protein, 18 aa, Artificial Sequence
  fusion protein
MGGKLSKKKKGYNVNDEK

SEQ ID NO: 9 - protein, 15 aa, Artificial Sequence
  fusion protein
MGGKLSKKKKGYNVN

SEQ ID NO: 10 - protein, 12 aa, Artificial Sequence
  fusion protein
MGGKLSKKKKGY

SEQ ID NO: 11 - protein, 11 aa, Artificial Sequence
  fusion protein
MGGKLSKKKKG

SEQ ID NO: 12 - protein, 10 aa, Artificial Sequence
  fusion protein
MGGKLSKKKK

SEQ ID NO: 13 - protein, 9 aa, Artificial Sequence
  fusion protein
MGGKLSKKK

SEQ ID NO: 14 - protein, 8 aa, Artificial Sequence
  fusion protein
MGGKLSKK

SEQ ID NO: 15 - protein, 7 aa, Artificial Sequence
  fusion protein
MGGKLSK

SEQ ID NO: 16 - protein, 8 aa, Artificial Sequence
  fusion protein
MGGKLAKK

SEQ ID NO: 17 - protein, 8 aa, Artificial Sequence
  fusion protein
MGGKFSKK

SEQ ID NO: 18 - protein, 8 aa, Artificial Sequence
  fusion protein
MGGKFAKK

SEQ ID NO: 19 - protein, 8 aa, Artificial Sequence
  fusion protein
MGGKSSKK

SEQ ID NO: 20 - protein, 8 aa, Artificial Sequence
  fusion protein
MGGKSAKK

SEQ ID NO: 21 - protein, 8 aa, Artificial Sequence
  fusion protein
MGGKQSKK

SEQ ID NO: 22 - protein, 8 aa, Artificial Sequence
  fusion protein
MGGKQAKK

SEQ ID NO: 23 - protein, 8 aa, Artificial Sequence
  fusion protein
MGGQLSKK

SEQ ID NO: 24 - protein, 8 aa, Artificial Sequence
  fusion protein
MGGQLAKK

SEQ ID NO: 25 - protein, 8 aa, Artificial Sequence
  fusion protein
MGGQFSKK

SEQ ID NO: 26 - protein, 8 aa, Artificial Sequence
  fusion protein
MGGQFAKK

SEQ ID NO: 27 - protein, 8 aa, Artificial Sequence
  fusion protein
MGGQSSKK

SEQ ID NO: 28 - protein, 8 aa, Artificial Sequence
  fusion protein
MGGQSAKK

SEQ ID NO: 29 - protein, 8 aa, Artificial Sequence
  fusion protein
MGGQQSKK

SEQ ID NO: 30 - protein, 8 aa, Artificial Sequence
  fusion protein
MGGQQAKK

SEQ ID NO: 31 - protein, 8 aa, Artificial Sequence
  fusion protein
MGAKLSKK

SEQ ID NO: 32 - protein, 8 aa, Artificial Sequence
  fusion protein
MGAKLAKK

SEQ ID NO: 33 - protein, 8 aa, Artificial Sequence
  fusion protein
MGAKFSKK

SEQ ID NO: 34 - protein, 8 aa, Artificial Sequence
  fusion protein
MGAKFAKK

SEQ ID NO: 35 - protein, 8 aa, Artificial Sequence
  fusion protein
MGAKSSKK

SEQ ID NO: 36 - protein, 8 aa, Artificial Sequence
  fusion protein
MGAKSAKK

SEQ ID NO: 37 - protein, 8 aa, Artificial Sequence
  fusion protein
MGAKQSKK

SEQ ID NO: 38 - protein, 8 aa, Artificial Sequence
  fusion protein
MGAKQAKK

SEQ ID NO: 39 - protein, 8 aa, Artificial Sequence
  fusion protein
MGAQLSKK

SEQ ID NO: 40 - protein, 8 aa, Artificial Sequence
  fusion protein
MGAQLAKK

SEQ ID NO: 41 - protein, 8 aa, Artificial Sequence
  fusion protein
MGAQFSKK

SEQ ID NO: 42 - protein, 8 aa, Artificial Sequence
  fusion protein
MGAQFAKK

SEQ ID NO: 43 - protein, 8 aa, Artificial Sequence
  fusion protein
MGAQSSKK

SEQ ID NO: 44 - protein, 8 aa, Artificial Sequence
  fusion protein
MGAQSAKK

SEQ ID NO: 45 - protein, 8 aa, Artificial Sequence
  fusion protein
MGAQQSKK

SEQ ID NO: 46 - protein, 8 aa, Artificial Sequence
  fusion protein
MGAQQAKK

SEQ ID NO: 47 - protein, 8 aa, Artificial Sequence
  fusion protein
MGSKLSKK

SEQ ID NO: 48 - protein, 8 aa, Artificial Sequence
  fusion protein
MGSKLAKK

SEQ ID NO: 49 - protein, 8 aa, Artificial Sequence
  fusion protein
MGSKFSKK

SEQ ID NO: 50 - protein, 8 aa, Artificial Sequence
  fusion protein
MGSKFAKK

SEQ ID NO: 51 - protein, 8 aa, Artificial Sequence
  fusion protein
MGSKSSKK

SEQ ID NO: 52 - protein, 8 aa, Artificial Sequence
  fusion protein
MGSKSAKK

SEQ ID NO: 53 - protein, 8 aa, Artificial Sequence
  fusion protein
MGSKQSKK

SEQ ID NO: 54 - protein, 8 aa, Artificial Sequence
  fusion protein
MGSKQAKK

SEQ ID NO: 55 - protein, 8 aa, Artificial Sequence
  fusion protein
MGSQLSKK

SEQ ID NO: 56 - protein, 8 aa, Artificial Sequence
  fusion protein
MGSQLAKK

SEQ ID NO: 57 - protein, 8 aa, Artificial Sequence
  fusion protein
MGSQFSKK

SEQ ID NO: 58 - protein, 8 aa, Artificial Sequence
  fusion protein
MGSQFAKK

SEQ ID NO: 59 - protein, 8 aa, Artificial Sequence
  fusion protein
MGSQSSKK

SEQ ID NO: 60 - protein, 8 aa, Artificial Sequence
  fusion protein
MGSQSAKK

SEQ ID NO: 61 - protein, 8 aa, Artificial Sequence
  fusion protein
MGSQQSKK

SEQ ID NO: 62 - protein, 8 aa, Artificial Sequence
  fusion protein
MGSQQAKK

SEQ ID NO: 63 - protein, 7 aa, Artificial Sequence
  fusion protein
MGGKLAK

SEQ ID NO: 64 - protein, 7 aa, Artificial Sequence
  fusion protein
MGGKFSK

SEQ ID NO: 65 - protein, 7 aa, Artificial Sequence
  fusion protein
MGGKFAK

SEQ ID NO: 66 - protein, 7 aa, Artificial Sequence
  fusion protein
MGGKSSK

SEQ ID NO: 67 - protein, 7 aa, Artificial Sequence
  fusion protein
MGGKSAK

SEQ ID NO: 68 - protein, 7 aa, Artificial Sequence
  fusion protein
MGGKQSK

SEQ ID NO: 69 - protein, 7 aa, Artificial Sequence
  fusion protein
MGGKQAK

SEQ ID NO: 70 - protein, 7 aa, Artificial Sequence
  fusion protein
MGGQLSK

SEQ ID NO: 71 - protein, 7 aa, Artificial Sequence
  fusion protein
MGGQLAK

SEQ ID NO: 72 - protein, 7 aa, Artificial Sequence
  fusion protein
MGGQFSK

SEQ ID NO: 73 - protein, 7 aa, Artificial Sequence
  fusion protein
MGGQFAK

SEQ ID NO: 74 - protein, 7 aa, Artificial Sequence
  fusion protein
MGGQSSK

SEQ ID NO: 75 - protein, 7 aa, Artificial Sequence
  fusion protein
MGGQSAK

SEQ ID NO: 76 - protein, 7 aa, Artificial Sequence
  fusion protein
MGGQQSK

SEQ ID NO: 77 - protein, 7 aa, Artificial Sequence
  fusion protein
MGGQQAK

SEQ ID NO: 78 - protein, 7 aa, Artificial Sequence
  fusion protein
MGAKLSK

SEQ ID NO: 79 - protein, 7 aa, Artificial Sequence
  fusion protein
MGAKLAK

SEQ ID NO: 80 - protein, 7 aa, Artificial Sequence
  fusion protein
MGAKFSK

SEQ ID NO: 81 - protein, 7 aa, Artificial Sequence
  fusion protein
MGAKFAK

SEQ ID NO: 82 - protein, 7 aa, Artificial Sequence
  fusion protein
MGAKSSK

SEQ ID NO: 83 - protein, 7 aa, Artificial Sequence
  fusion protein
MGAKSAK

SEQ ID NO: 84 - protein, 7 aa, Artificial Sequence
  fusion protein
MGAKQSK

SEQ ID NO: 85 - protein, 7 aa, Artificial Sequence
  fusion protein
MGAKQAK

SEQ ID NO: 86 - protein, 7 aa, Artificial Sequence
  fusion protein
MGAQLSK

SEQ ID NO: 87 - protein, 7 aa, Artificial Sequence
  fusion protein
MGAQLAK

SEQ ID NO: 88 - protein, 7 aa, Artificial Sequence
  fusion protein
MGAQFSK

SEQ ID NO: 89 - protein, 7 aa, Artificial Sequence
  fusion protein
MGAQFAK

SEQ ID NO: 90 - protein, 7 aa, Artificial Sequence
  fusion protein
MGAQSSK

SEQ ID NO: 91 - protein, 7 aa, Artificial Sequence
  fusion protein
MGAQSAK

SEQ ID NO: 92 - protein, 7 aa, Artificial Sequence
  fusion protein
MGAQQSK

SEQ ID NO: 93 - protein, 7 aa, Artificial Sequence
  fusion protein
MGAQQAK

SEQ ID NO: 94 - protein, 7 aa, Artificial Sequence
  fusion protein
MGSKLSK

SEQ ID NO: 95 - protein, 7 aa, Artificial Sequence
  fusion protein
MGSKLAK

SEQ ID NO: 96 - protein, 7 aa, Artificial Sequence
  fusion protein
MGSKFSK

SEQ ID NO: 97 - protein, 7 aa, Artificial Sequence
  fusion protein
MGSKFAK

SEQ ID NO: 98 - protein, 7 aa, Artificial Sequence
  fusion protein
MGSKSSK

SEQ ID NO: 99 - protein, 7 aa, Artificial Sequence
  fusion protein
MGSKSAK

SEQ ID NO: 100 - protein, 7 aa, Artificial Sequence
  fusion protein
MGSKQSK

SEQ ID NO: 101 - protein, 7 aa, Artificial Sequence
  fusion protein
MGSKQAK

SEQ ID NO: 102 - protein, 7 aa, Artificial Sequence
  fusion protein
MGSQLSK

SEQ ID NO: 103 - protein, 7 aa, Artificial Sequence
  fusion protein
MGSQLAK

SEQ ID NO: 104 - protein, 7 aa, Artificial Sequence
  fusion protein
MGSQFSK

SEQ ID NO: 105 - protein, 7 aa, Artificial Sequence
  fusion protein
MGSQFAK

SEQ ID NO: 106 - protein, 7 aa, Artificial Sequence
  fusion protein
MGSQSSK

SEQ ID NO: 107 - protein, 7 aa, Artificial Sequence
  fusion protein
MGSQSAK

SEQ ID NO: 108 - protein, 7 aa, Artificial Sequence
  fusion protein
MGSQQSK

SEQ ID NO: 109 - protein, 7 aa, Artificial Sequence
  fusion protein
MGSQQAK

SEQ ID NO: 110 - protein, 9 aa, Artificial Sequence
  scaffold protein
MGAKLSKKK

SEQ ID NO: 111 - protein, 167 aa, Artificial Sequence
  scaffold protein
MGGKLSKKKKGYNVNDEKAKEKDKKAEGAASGGSGGSDYKDDDDKGGGSGMASNFTQFVLVDNGGTGDVTVAPSNFANGIAEWISSNSRSQAYKVTCSVRQSSAQNRKYTIKVEVPKGAWRSYLNMELTIPIFATNSDCELIVKAMQGLLKDGNPIPSAIAANSGIY

SEQ ID NO: 112 - protein, 167 aa, Artificial Sequence
  scaffold protein
MGGKLSKKKKGYNVNDEKAKEKDKKAEGAASGGSGGSDYKDDDDKGGGSGMASNFTQFVLVDNGGTGDVTVAPSNFANGIAEWISSNSRSQAYKVTCSVRQSSAQKRKYTIKVEVPKGAWRSYLNMELTIPIFATNSDCELIVKAMQGLLKDGNPIPSAIAANSGIY

SEQ ID NO: 113 - protein, 296 aa, Artificial Sequence
  scaffold protein
MGGKLSKKKKGYNVNDEKAKEKDKKAEGAASGGSGGSDYKDDDDKGGGSGMASNFTQFVLVDNGGTGDVTVAPSNFANGIAEWISSNSRSQAYKVTCSVRQSSAQNRKYTIKVEVPKGAWRSYLNMELTIPIFATNSDCELIVKAMQGLLKDGNPIPSAIAANSGIYGSGGSGGSGGSGMASNFTQFVLVDNGGTGDVTVAPSNFANGIAEWISSNSRSQAYKVTCSVRQSSAQNRKYTIKVEVPKGAWRSYLNMELTIPIFATNSDCELIVKAMQGLLKDGNPIPSAIAANSGIY

SEQ ID NO: 114 - protein, 296 aa, Artificial Sequence
  scaffold protein
MGGKLSKKKKGYNVNDEKAKEKDKKAEGAASGGSGGSDYKDDDDKGGGSGMASNFTQFVLVDNGGTGDVTVAPSNFANGIAEWISSNSRSQAYKVTCSVRQSSAQKRKYTIKVEVPKGAWRSYLNMELTIPIFATNSDCELIVKAMQGLLKDGNPIPSAIAANSGIYGSGGSGGSGGSGMASNFTQFVLVDNGGTGDVTVAPSNFANGIAEWISSNSRSQAYKVTCSVRQSSAQKRKYTIKVEVPKGAWRSYLNMELTIPIFATNSDCELIVKAMQGLLKDGNPIPSAIAANSGIY

SEQ ID NO: 115 - RNA, 680 nt, Artificial Sequence
  scaffold protein
augaagcccaccgagaacaacgaagacuucaacaucguggccguggccagcaacuucgcgaccacggaucucgaugcugaccgcgggaaguugcccggcaagaagcugccgcuggaggugcucaaagaguuggaagccaaugcccggaaagcuggcugcaccaggggcugucugaucugccugucccacaucaagugcacgcccaagaugaagaaguucaucccaggacgcugccacaccuacgaaggcgacaaagaguccgcacagggcggcauaggcgaggcgaucgucgacauuccugagauuccuggguucaaggacuuggagcccuuggagcaguucaucgcacaggucgaucuguguguggacugcacaacuggcugccucaaagggcuugccaacgugcaguguucugaccugcucaagaaguggcugccgcaacgcugugcgaccuuugccagcaagauccagggccagguggacaagaucaagggggccgguggugacuaaggauccaucgauaagcuucaucgaaacaugaggaucacccauaucugcagucgacaucgaaacaugaggaucacccaugucugcagucgacaucgaaacaugaggaucacccaugucugcagucgacaucgaaacaugaggaucacccaugucugcagucgacaucgaaa

SEQ ID NO: 116 - protein, 9 aa, Artificial Sequence
  scaffold peptide
  misc_feature (3)..(3): Xaa can be any naturally occurring amino acid
MGXKLSKKK

SEQ ID NO: 117 - protein, 9 aa, Artificial Sequence
  scaffold peptide
  misc_feature (3)..(3): Xaa can be any naturally occurring amino acid
MGXKLSKKK

SEQ ID NO: 118 - protein, 8 aa, Artificial Sequence
  scaffold protein
  MISC_FEATURE (3)..(3): Xaa = G, A, S
  MISC_FEATURE (4)..(3): Xaa = K, Q
  misc_feature (4)..(4): Xaa can be any naturally occurring amino acid
  MISC_FEATURE (5)..(5): Xaa = L, F, S, Q
  MISC_FEATURE (6)..(6): Xaa = S, A
MGXXXXKK

SEQ ID NO: 119 - DNA, 20 bp, Artificial Sequence
  scaffold protein
tggaggtgctcaaagagttg

SEQ ID NO: 120 - DNA, 17 bp, Artificial Sequence
  scaffold protein
ttgggcgtgcacttgat

SEQ ID NO: 121 - DNA, 13 bp, Artificial Sequence
  scaffold protein
gggcattggcttc

SEQ ID NO: 122 - protein, 60 aa, Artificial Sequence
  scaffold protein
MGGKLSKKKKGYNVNDEKAKEKDKKAEGAASAGGGGSDYKDDDDKGGGGSVSKGEELFTG

SEQ ID NO: 123 - protein, 60 aa, Artificial Sequence
  scaffold protein
MAGKLSKKKKGYNVNDEKAKEKDKKAEGAASAGGGGSDYKDDDDKGGGGSVSKGEELFTG

SEQ ID NO: 124 - protein, 60 aa, Artificial Sequence
  scaffold protein
MGAKLSKKKKGYNVNDEKAKEKDKKAEGAASAGGGGSDYKDDDDKGGGGSVSKGEELFTG

SEQ ID NO: 125 - protein, 60 aa, Artificial Sequence
  scaffold protein
MAAKLSKKKKGYNVNDEKAKEKDKKAEGAASAGGGGSDYKDDDDKGGGGSVSKGEELFTG

SEQ ID NO: 126 - protein, 57 aa, Artificial Sequence
  scaffold protein
MGGKLSKKKKGYNVNDEKAKEKDKKAESAGGGGSDYKDDDDKGGGGSVSKGEELFTG

SEQ ID NO: 127 - protein, 54 aa, Artificial Sequence
  scaffold protein
MGGKLSKKKKGYNVNDEKAKEKDKSAGGGGSDYKDDDDKGGGGSVSKGEELFTG

SEQ ID NO: 128 - protein, 51 aa, Artificial Sequence
  scaffold protein
MGGKLSKKKKGYNVNDEKAKESAGGGGSDYKDDDDKGGGGSVSKGEELFTG

SEQ ID NO: 129 - protein, 48 aa, Artificial Sequence
  scaffold protein
MGGKLSKKKKGYNVNDEKSAGGGGSDYKDDDDKGGGGSVSKGEELFTG

SEQ ID NO: 130 - protein, 45 aa, Artificial Sequence
  scaffold protein
MGGKLSKKKKGYNVNSAGGGGSDYKDDDDKGGGGSVSKGEELFTG

SEQ ID NO: 131 - protein, 42 aa, Artificial Sequence
  scaffold protein
MGGKLSKKKKGYSAGGGGSDYKDDDDKGGGGSVSKGEELFTG

SEQ ID NO: 132 - protein, 39 aa, Artificial Sequence
  scaffold protein
MGGKLSKKKSAGGGGSDYKDDDDKGGGGSVSKGEELFTG

SEQ ID NO: 133 - protein, 36 aa, Artificial Sequence
  scaffold protein
MGGKLSSAGGGGSDYKDDDDKGGGGSVSKGEELFTG

SEQ ID NO: 134 - protein, 33 aa, Artificial Sequence
  scaffold protein
MGGSAGGGGSDYKDDDDKGGGGSVSKGEELFTG

SEQ ID NO: 135 - protein, 54 aa, Artificial Sequence
  scaffold protein
MGGKLSKKKKGYNVNDEKAKEKDKKAEGAASAGGGGSDYKDDDDKGGGGSVSKG

SEQ ID NO: 136 - protein, 36 aa, Artificial Sequence
  scaffold protein
MGGKLSKKKKGYSAGGGGSDYKDDDDKGGGGSVSKG

SEQ ID NO: 137 - protein, 35 aa, Artificial Sequence
  scaffold protein
MGGKLSKKKKGSAGGGGSDYKDDDDKGGGGSVSKG

SEQ ID NO: 138 - protein, 34 aa, Artificial Sequence
  scaffold protein
MGGKLSKKKKSAGGGGSDYKDDDDKGGGGSVSKG

SEQ ID NO: 139 - protein, 33 aa, Artificial Sequence
  scaffold protein
MGGKLSKKKSAGGGGSDYKDDDDKGGGGSVSKG

SEQ ID NO: 140 - protein, 32 aa, Artificial Sequence
  scaffold protein
MGGKLSKKSAGGGGSDYKDDDDKGGGGSVSKG

SEQ ID NO: 141 - protein, 31 aa, Artificial Sequence
  scaffold protein
MGGKLSKSAGGGGSDYKDDDDKGGGGSVSKG

SEQ ID NO: 142 - protein, 30 aa, Artificial Sequence
  scaffold protein
MGGKLSSAGGGGSDYKDDDDKGGGGSVSKG

SEQ ID NO: 143 - protein, 30 aa, Artificial Sequence
  scaffold protein
MGGKLDKKKKGYNVNDEKAKEKDKKAEGAA

SEQ ID NO: 144 - protein, 30 aa, Artificial Sequence
  scaffold protein
MGGKLAKKKKGYNVNDEKAKEKDKKAEGAA

SEQ ID NO: 145 - protein, 30 aa, Artificial Sequence
  scaffold protein
MGGKQSKKKKGYNVNDEKAKEKDKKAEGAA

SEQ ID NO: 146 - protein, 30 aa, Artificial Sequence
  scaffold protein
MGAKKKKKRFSFKKSFKLSGFSFKKNKKEA

SEQ ID NO: 147 - protein, 30 aa, Artificial Sequence
  scaffold protein
MAAKKKKKRFSFKKSFKLSGFSFKKNKKEA

SEQ ID NO: 148 - protein, 30 aa, Artificial Sequence
  scaffold protein
MGAKKSKKRFSFKKSFKLSGFSFKKNKKEA

SEQ ID NO: 149 - protein, 30 aa, Artificial Sequence
  scaffold protein
MGAKKAKKRFSFKKPFKLSGFSFKKNKKEA

SEQ ID NO: 150 - protein, 153 aa, Artificial Sequence
  scaffold protein
MGGKLSKKKKSAGGSGGSTSGSGDYKDDDDKGSGFEMDQVQLVESGGALVQPGGSLRLSCAASGFPVNRYSMRWYRQAPGKEREWVAGMSSAGDRSSYEDSVKGRFTISRDDARNTVYLQMNSLKPEDTAVYYCNVNVGFEYWGQGTQVTVSS

SEQ ID NO: 151 - protein, 4 aa, Artificial Sequence
  effector domain
KKKK

SEQ ID NO: 152 - protein, 5 aa, Artificial Sequence
  effector domain
KKKKK

SEQ ID NO: 153 - protein, 4 aa, Artificial Sequence
  effector domain
RRRR

SEQ ID NO: 154 - protein, 5 aa, Artificial Sequence
  effector domain
RRRRR

SEQ ID NO: 155 - protein, 4 aa, Artificial Sequence
  effector domain
  MISC_FEATURE (1)..(4): Xaa = K, R
XXXX

SEQ ID NO: 156 - protein, 5 aa, Artificial Sequence
  effector domain
  MISC_FEATURE (1)..(5): Xaa= K, R
XXXXX

SEQ ID NO: 157 - protein, 7 aa, Artificial Sequence
  scaffold protein
GGKLSKK

SEQ ID NO: 158 - protein, 7 aa, Artificial Sequence
  scaffold protein
GAKLSKK

SEQ ID NO: 159 - protein, 7 aa, Artificial Sequence
  scaffold protein
GGKQSKK

SEQ ID NO: 160 - protein, 7 aa, Artificial Sequence
  scaffold protein
GGKLAKK

SEQ ID NO: 161 - protein, 8 aa, Artificial Sequence
  scaffold protein
GGKLSKKK

SEQ ID NO: 162 - protein, 8 aa, Artificial Sequence
  scaffold protein
GGKLSKKS

SEQ ID NO: 163 - protein, 8 aa, Artificial Sequence
  scaffold protein
GAKLSKKK

SEQ ID NO: 164 - protein, 8 aa, Artificial Sequence
  scaffold protein
GAKLSKKS

SEQ ID NO: 165 - protein, 8 aa, Artificial Sequence
  scaffold protein
GGKQSKKK

SEQ ID NO: 166 - protein, 8 aa, Artificial Sequence
  scaffold protein
GGKQSKKS

SEQ ID NO: 167 - protein, 8 aa, Artificial Sequence
  scaffold protein
GGKLAKKK

SEQ ID NO: 168 - protein, 8 aa, Artificial Sequence
  scaffold protein
GGKLAKKS

SEQ ID NO: 169 - protein, 14 aa, Artificial Sequence
  scaffold protein
GGKLSKKKKGYNVN

SEQ ID NO: 170 - protein, 14 aa, Artificial Sequence
  scaffold protein
GAKLSKKKKGYNVN

SEQ ID NO: 171 - protein, 14 aa, Artificial Sequence
  scaffold protein
GGKQSKKKKGYNVN

SEQ ID NO: 172 - protein, 14 aa, Artificial Sequence
  scaffold protein
GGKLAKKKKGYNVN

SEQ ID NO: 173 - protein, 14 aa, Artificial Sequence
  scaffold protein
GGKLSKKKKGYSGG

SEQ ID NO: 174 - protein, 14 aa, Artificial Sequence
  scaffold protein
GGKLSKKKKGSGGS

SEQ ID NO: 175 - protein, 14 aa, Artificial Sequence
  scaffold protein
GGKLSKKKKSGGSG

SEQ ID NO: 176 - protein, 14 aa, Artificial Sequence
  scaffold protein
GGKLSKKKSGGSGG

SEQ ID NO: 177 - protein, 14 aa, Artificial Sequence
  scaffold protein
GGKLSKKSGGSGGS

SEQ ID NO: 178 - protein, 14 aa, Artificial Sequence
  scaffold protein
GGKLSKSGGSGGSV

SEQ ID NO: 179 - protein, 14 aa, Artificial Sequence
  scaffold protein
GAKKSKKRFSFKKS

SEQ ID NO: 180 - protein, 8 aa, Artificial Sequence
  scaffold protein
  MISC_FEATURE (4)..(4): Xaa= K, Q
  MISC_FEATURE (5)..(5): Xaa= L, F, S, Q
  MISC_FEATURE (6)..(6): Xaa= S, A
MGGXXXKK

SEQ ID NO: 181 - protein, 8 aa, Artificial Sequence
  scaffold protein
  MISC_FEATURE (4)..(4): Xaa= K, Q
  MISC_FEATURE (5)..(5): Xaa= L, F, S, Q
  MISC_FEATURE (6)..(6): Xaa= S, A
MGAXXXKK

SEQ ID NO: 182 - protein, 8 aa, Artificial Sequence
  scaffold protein
  MISC_FEATURE (4)..(4): Xaa = K, Q
  MISC_FEATURE (5)..(5): Xaa = L, F, S, Q
  MISC_FEATURE (6)..(6): Xaa = S, A
MGSXXXKK

SEQ ID NO: 183 - protein, 8 aa, Artificial Sequence
  scaffold protein
  MISC_FEATURE (3)..(3): Xaa = G, A, S
  MISC_FEATURE (5)..(5): Xaa = L, F, S, Q
  MISC_FEATURE (6)..(6): Xaa = S, A
MGXKXXKK

SEQ ID NO: 184 - protein, 8 aa, Artificial Sequence
  scaffold protein
  MISC_FEATURE (3)..(3): Xaa= G, A, S
  MISC_FEATURE (5)..(5): Xaa= L, F, S, Q
  MISC_FEATURE (6)..(6): Xaa= S, A
MGXQXXKK

SEQ ID NO: 185 - protein, 8 aa, Artificial Sequence
  scaffold protein
  MISC_FEATURE (3)..(3): Xaa = G, A, S
  MISC_FEATURE (4)..(4): Xaa = K, Q
  MISC_FEATURE (6)..(6): Xaa = S, A
MGXXLXKK

SEQ ID NO: 186 - protein, 8 aa, Artificial Sequence
  scaffold protein
  MISC_FEATURE (3)..(3): Xaa = G, A, S
  MISC_FEATURE (4)..(4): Xaa = K, Q
  MISC_FEATURE (6)..(6): Xaa = S, A
MGXXFXKK

SEQ ID NO: 187 - protein, 8 aa, Artificial Sequence
  scaffold protein
  MISC_FEATURE (3)..(3): Xaa = G, A, S
  MISC_FEATURE (4)..(4): Xaa = K, Q
  MISC_FEATURE (6)..(6): Xaa = S, A
MGXXSXKK

SEQ ID NO: 188 - protein, 8 aa, Artificial Sequence
  scaffold protein
  MISC_FEATURE (3)..(3): Xaa = G, A, S
  MISC_FEATURE (4)..(4): Xaa = K, Q
  MISC_FEATURE (6)..(6): Xaa = S, A
MGXXQXKK

SEQ ID NO: 189 - protein, 8 aa, Artificial Sequence
  scaffold protein
  MISC_FEATURE (3)..(3): Xaa= G, A, S
  MISC_FEATURE (4)..(4): Xaa= K, Q
  MISC_FEATURE (5)..(5): Xaa= L, F, S, Q
MGXXXSKK

SEQ ID NO: 190 - protein, 8 aa, Artificial Sequence
  scaffold protein
  MISC_FEATURE (3)..(3): Xaa = G, A, S
  MISC_FEATURE (4)..(4): Xaa = K, Q
  MISC_FEATURE (5)..(5): Xaa = L, F, S, Q
MGXXXAKK

SEQ ID NO: 191 - protein, 7 aa, Artificial Sequence
  scaffold protein
  MISC_FEATURE (3)..(3): Xaa = K, Q
  MISC_FEATURE (4)..(4): Xaa = L, F, S, Q
  MISC_FEATURE (5)..(5): Xaa = S, A
GGXXXKK

SEQ ID NO: 192 - protein, 7 aa, Artificial Sequence
  scaffold protein
  MISC_FEATURE (3)..(3): Xaa = K, Q
  MISC_FEATURE (4)..(4): Xaa = L, F, S, Q
  MISC_FEATURE (5)..(5): Xaa = S, A
GAXXXKK

SEQ ID NO: 193 - protein, 7 aa, Artificial Sequence
  scaffold protein
  MISC_FEATURE (3)..(3): Xaa = K, Q
  MISC_FEATURE (4)..(4): Xaa = L, F, S, Q
  MISC_FEATURE (5)..(5): Xaa = S, A
GSXXXKK

SEQ ID NO: 194 - protein, 7 aa, Artificial Sequence
  scaffold protein
  MISC_FEATURE (2)..(2): Xaa = G, A, S
  MISC_FEATURE (4)..(4): Xaa = L, F, S, Q
  MISC_FEATURE (5)..(5): Xaa = S, A
GXKXXKK

SEQ ID NO: 195 - protein, 7 aa, Artificial Sequence
  scaffold protein
  MISC_FEATURE (2)..(2): Xaa = G, A, S
  MISC_FEATURE (4)..(4): Xaa = L, F, S, Q
  MISC_FEATURE (5)..(5): Xaa = S, A
GXQXXKK

SEQ ID NO: 196 - protein, 7 aa, Artificial Sequence
  scaffold protein
  MISC_FEATURE (2)..(2): Xaa= G, A, S
  MISC_FEATURE (3)..(3): Xaa= K, Q
  MISC_FEATURE (5)..(5): Xaa= S, A
GXXLXKK

SEQ ID NO: 197 - protein, 7 aa, Artificial Sequence
  scaffold protein
  MISC_FEATURE (2)..(2): Xaa = G, A, S
  MISC_FEATURE (3)..(3): Xaa = K, Q
  MISC_FEATURE (5)..(5): Xaa = S, A
GXXFXKK

SEQ ID NO: 198 - protein, 7 aa, Artificial Sequence
  scaffold protein
  MISC_FEATURE (2)..(2): Xaa = G, A, S
  MISC_FEATURE (3)..(3): Xaa = K, Q
  MISC_FEATURE (5)..(5): Xaa = S, A
GXXSXKK

SEQ ID NO: 199 - protein, 7 aa, Artificial Sequence
  scaffold protein
  MISC_FEATURE (2)..(2): Xaa = G, A, S
  MISC_FEATURE (3)..(3): Xaa = K, Q
  MISC_FEATURE (5)..(5): Xaa = S, A
GXXQXKK

SEQ ID NO: 200 - protein, 7 aa, Artificial Sequence
  scaffold protein
  MISC_FEATURE (2)..(2): Xaa = G, A, S
  MISC_FEATURE (3)..(3): Xaa = K, Q
  MISC_FEATURE (4)..(4): Xaa = L, F, S, Q
GXXXSKK

SEQ ID NO: 201 - protein, 7 aa, Artificial Sequence
  scaffold protein
  MISC_FEATURE (2)..(2): Xaa = G, A, S
  MISC_FEATURE (3)..(3): Xaa = K, Q
  MISC_FEATURE (4)..(4): Xaa = L, F, S, Q
GXXXAKK

SEQ ID NO: 202 - protein, 7 aa, Artificial Sequence
  scaffold protein
  MISC_FEATURE (2)..(2): Xaa = G, A, S
  MISC_FEATURE (3)..(3): Xaa = K, Q
  MISC_FEATURE (4)..(4): Xaa = L, F, S, Q
  MISC_FEATURE (5)..(5): Xaa = S, A
GXXXXKK

SEQ ID NO: 203 - protein, 6 aa, Artificial Sequence
  N-terminus domain
GGKLSK

SEQ ID NO: 204 - protein, 6 aa, Artificial Sequence
  N-terminus domain
GAKLSK

SEQ ID NO: 205 - protein, 6 aa, Artificial Sequence
  N-terminus domain
GGKQSK

SEQ ID NO: 206 - protein, 6 aa, Artificial Sequence
  N-terminus domain
GGKLAK

SEQ ID NO: 207 - protein, 4 aa, Artificial Sequence
  N-terminus domain
KKKG

SEQ ID NO: 208 - protein, 5 aa, Artificial Sequence
  N-terminus domain
KKKGY

SEQ ID NO: 209 - protein, 6 aa, Artificial Sequence
  N-terminus domain
KKKGYN

SEQ ID NO: 210 - protein, 7 aa, Artificial Sequence
  N-terminus domain
KKKGYNV

SEQ ID NO: 211 - protein, 8 aa, Artificial Sequence
  N-terminus domain
KKKGYNVN

SEQ ID NO: 212 - protein, 6 aa, Artificial Sequence
  N-terminus domain
KKKGYS

SEQ ID NO: 213 - protein, 6 aa, Artificial Sequence
  N-terminus domain
KKKGYG

SEQ ID NO: 214 - protein, 7 aa, Artificial Sequence
  N-terminus domain
KKKGYGG

SEQ ID NO: 215 - protein, 5 aa, Artificial Sequence
  N-terminus domain
KKKGS

SEQ ID NO: 216 - protein, 6 aa, Artificial Sequence
  N-terminus domain
KKKGSG

SEQ ID NO: 217 - protein, 6 aa, Artificial Sequence
  N-terminus domain
KKKGSG

SEQ ID NO: 218 - protein, 7 aa, Artificial Sequence
  N-terminus domain
KKKGSGS

SEQ ID NO: 219 - protein, 4 aa, Artificial Sequence
  N-terminus domain
KKKS

SEQ ID NO: 220 - protein, 5 aa, Artificial Sequence
  N-terminus domain
KKKSG

SEQ ID NO: 221 - protein, 6 aa, Artificial Sequence
  N-terminus domain
KKKSGG

SEQ ID NO: 222 - protein, 7 aa, Artificial Sequence
  N-terminus domain
KKKSGGS

SEQ ID NO: 223 - protein, 8 aa, Artificial Sequence
  N-terminus domain
KKKSGGSG

SEQ ID NO: 224 - protein, 8 aa, Artificial Sequence
  N-terminus domain
KKSGGSGG

SEQ ID NO: 225 - protein, 10 aa, Artificial Sequence
  N-terminus domain
KKKSGGSGGS

SEQ ID NO: 226 - protein, 8 aa, Artificial Sequence
  N-terminus domain
KRFSFKKS

SEQ ID NO: 227 - protein, 29 aa, Artificial Sequence
  Scaffold Protein
GGKLSKKKKGYNVNDEKAKEKDKKAEGAA

SEQ ID NO: 228 - protein, 28 aa, Artificial Sequence
  Scaffold Protein
GGKLSKKKKGYNVNDEKAKEKDKKAEGA

SEQ ID NO: 229 - protein, 27 aa, Artificial Sequence
  Scaffold Protein
GGKLSKKKKGYNVNDEKAKEKDKKAEG

SEQ ID NO: 230 - protein, 26 aa, Artificial Sequence
  Scaffold Protein
GGKLSKKKKGYNVNDEKAKEKDKKAE

SEQ ID NO: 231 - protein, 25 aa, Artificial Sequence
  Scaffold Protein
GGKLSKKKKGYNVNDEKAKEKDKKA

SEQ ID NO: 232 - protein, 24 aa, Artificial Sequence
  Scaffold Protein
GGKLSKKKKGYNVNDEKAKEKDKK

SEQ ID NO: 233 - protein, 23 aa, Artificial Sequence
  Scaffold Protein
GGKLSKKKKGYNVNDEKAKEKDK

SEQ ID NO: 234 - protein, 22 aa, Artificial Sequence
  Scaffold Protein
GGKLSKKKKGYNVNDEKAKEKD

SEQ ID NO: 235 - protein, 21 aa, Artificial Sequence
  Scaffold Protein
GGKLSKKKKGYNVNDEKAKEK

SEQ ID NO: 236 - protein, 20 aa, Artificial Sequence
  Scaffold Protein
GGKLSKKKKGYNVNDEKAKE

SEQ ID NO: 237 - protein, 19 aa, Artificial Sequence
  Scaffold Protein
GGKLSKKKKGYNVNDEKAK

SEQ ID NO: 238 - protein, 18 aa, Artificial Sequence
  Scaffold Protein
GGKLSKKKKGYNVNDEKA

SEQ ID NO: 239 - protein, 17 aa, Artificial Sequence
  Scaffold Protein
GGKLSKKKKGYNVNDEK

SEQ ID NO: 240 - protein, 16 aa, Artificial Sequence
  Scaffold Protein
GGKLSKKKKGYNVNDE

SEQ ID NO: 241 - protein, 15 aa, Artificial Sequence
  Scaffold Protein
GGKLSKKKKGYNVND

SEQ ID NO: 242 - protein, 13 aa, Artificial Sequence
  Scaffold Protein
GGKLSKKKKGYNV

SEQ ID NO: 243 - protein, 12 aa, Artificial Sequence
  Scaffold Protein
GGKLSKKKKGYN

SEQ ID NO: 244 - protein, 11 aa, Artificial Sequence
  Scaffold Protein
GGKLSKKKKGY

SEQ ID NO: 245 - protein, 10 aa, Artificial Sequence
  Scaffold Protein
GGKLSKKKKG

SEQ ID NO: 246 - protein, 9 aa, Artificial Sequence
  Scaffold Protein
GGKLSKKKK

SEQ ID NO: 247 - protein, 29 aa, Artificial Sequence
  Scaffold Protein
GAKKSKKRFSFKKSFKLSGFSFKKNKKEA

SEQ ID NO: 248 - protein, 28 aa, Artificial Sequence
  Scaffold Protein
GAKKSKKRFSFKKSFKLSGFSFKKNKKE

SEQ ID NO: 249 - protein, 27 aa, Artificial Sequence
  Scaffold Protein
GAKKSKKRFSFKKSFKLSGFSFKKNKK

SEQ ID NO: 250 - protein, 26 aa, Artificial Sequence
  Scaffold Protein
GAKKSKKRFSFKKSFKLSGFSFKKNK

SEQ ID NO: 251 - protein, 25 aa, Artificial Sequence
  Scaffold Protein
GAKKSKKRFSFKKSFKLSGFSFKKN

SEQ ID NO: 252 - protein, 24 aa, Artificial Sequence
  Scaffold Protein
GAKKSKKRFSFKKSFKLSGFSFKK

SEQ ID NO: 253 - protein, 23 aa, Artificial Sequence
  Scaffold Protein
GAKKSKKRFSFKKSFKLSGFSFK

SEQ ID NO: 254 - protein, 22 aa, Artificial Sequence
  Scaffold Protein
GAKKSKKRFSFKKSFKLSGFSF

SEQ ID NO: 255 - protein, 21 aa, Artificial Sequence
  Scaffold Protein
GAKKSKKRFSFKKSFKLSGFS

SEQ ID NO: 256 - protein, 20 aa, Artificial Sequence
  Scaffold Protein
GAKKSKKRFSFKKSFKLSGF

SEQ ID NO: 257 - protein, 19 aa, Artificial Sequence
  Scaffold Protein
GAKKSKKRFSFKKSFKLSG

SEQ ID NO: 258 - protein, 18 aa, Artificial Sequence
  Scaffold Protein
GAKKSKKRFSFKKSFKLS

SEQ ID NO: 259 - protein, 17 aa, Artificial Sequence
  Scaffold Protein
GAKKSKKRFSFKKSFKL

SEQ ID NO: 260 - protein, 16 aa, Artificial Sequence
  Scaffold Protein
GAKKSKKRFSFKKSFK

SEQ ID NO: 261 - protein, 15 aa, Artificial Sequence
  Scaffold Protein
GAKKSKKRFSFKKSF

SEQ ID NO: 262 - protein, 13 aa, Artificial Sequence
  Scaffold Protein
GAKKSKKRFSFKK

SEQ ID NO: 263 - protein, 12 aa, Artificial Sequence
  Scaffold Protein
GAKKSKKRFSFK

SEQ ID NO: 264 - protein, 11 aa, Artificial Sequence
  Scaffold Protein
GAKKSKKRFSF

SEQ ID NO: 265 - protein, 10 aa, Artificial Sequence
  Scaffold Protein
GAKKSKKRFS

SEQ ID NO: 266 - protein, 9 aa, Artificial Sequence
  Scaffold Protein
GAKKSKKRF

SEQ ID NO: 267 - protein, 8 aa, Artificial Sequence
  Scaffold Protein
GAKKSKKR

SEQ ID NO: 268 - protein, 7 aa, Artificial Sequence
  Scaffold Protein
GAKKSKK

SEQ ID NO: 269 - protein, 29 aa, Artificial Sequence
  Scaffold Protein
GAKKAKKRFSFKKSFKLSGFSFKKNKKEA

SEQ ID NO: 270 - protein, 28 aa, Artificial Sequence
  Scaffold Protein
GAKKAKKRFSFKKSFKLSGFSFKKNKKE

SEQ ID NO: 271 - protein, 27 aa, Artificial Sequence
  Scaffold Protein
GAKKAKKRFSFKKSFKLSGFSFKKNKK

SEQ ID NO: 272 - protein, 26 aa, Artificial Sequence
  Scaffold Protein
GAKKAKKRFSFKKSFKLSGFSFKKNK

SEQ ID NO: 273 - protein, 25 aa, Artificial Sequence
  Scaffold Protein
GAKKAKKRFSFKKSFKLSGFSFKKN

SEQ ID NO: 274 - protein, 24 aa, Artificial Sequence
  Scaffold Protein
GAKKAKKRFSFKKSFKLSGFSFKK

SEQ ID NO: 275 - protein, 23 aa, Artificial Sequence
  Scaffold Protein
GAKKAKKRFSFKKSFKLSGFSFK

SEQ ID NO: 276 - protein, 22 aa, Artificial Sequence
  Scaffold Protein
GAKKAKKRFSFKKSFKLSGFSF

SEQ ID NO: 277 - protein, 21 aa, Artificial Sequence
  Scaffold Protein
GAKKAKKRFSFKKSFKLSGFS

SEQ ID NO: 278 - protein, 20 aa, Artificial Sequence
  Scaffold Protein
GAKKAKKRFSFKKSFKLSGF

SEQ ID NO: 279 - protein, 19 aa, Artificial Sequence
  Scaffold Protein
GAKKAKKRFSFKKSFKLSG

SEQ ID NO: 280 - protein, 18 aa, Artificial Sequence
  Scaffold Protein
GAKKAKKRFSFKKSFKLS

SEQ ID NO: 281 - protein, 17 aa, Artificial Sequence
  Scaffold Protein
GAKKAKKRFSFKKSFKL

SEQ ID NO: 282 - protein, 16 aa, Artificial Sequence
  Scaffold Protein
GAKKAKKRFSFKKSFK

SEQ ID NO: 283 - protein, 15 aa, Artificial Sequence
  Scaffold Protein
GAKKAKKRFSFKKSF

SEQ ID NO: 284 - protein, 14 aa, Artificial Sequence
  Scaffold Protein
GAKKAKKRFSFKKS

SEQ ID NO: 285 - protein, 13 aa, Artificial Sequence
  Scaffold Protein
GAKKAKKRFSFKK

SEQ ID NO: 286 - protein, 12 aa, Artificial Sequence
  Scaffold Protein
GAKKAKKRFSFK

SEQ ID NO: 287 - protein, 11 aa, Artificial Sequence
  Scaffold Protein
GAKKAKKRFSF

SEQ ID NO: 288 - protein, 10 aa, Artificial Sequence
  Scaffold Protein
GAKKAKKRFS

SEQ ID NO: 289 - protein, 9 aa, Artificial Sequence
  Scaffold Protein
GAKKAKKRF

SEQ ID NO: 290 - protein, 8 aa, Artificial Sequence
  Scaffold Protein
GAKKAKKR

SEQ ID NO: 291 - protein, 7 aa, Artificial Sequence
  Scaffold Protein
GAKKAKK

SEQ ID NO: 292 - protein, 28 aa, Artificial Sequence
  Scaffold Protein
GAQESKKKKKKRFSFKKSFKLSGFSFKK

SEQ ID NO: 293 - protein, 27 aa, Artificial Sequence
  Scaffold Protein
GAQESKKKKKKRFSFKKSFKLSGFSFK

SEQ ID NO: 294 - protein, 26 aa, Artificial Sequence
  Scaffold Protein
GAQESKKKKKKRFSFKKSFKLSGFSF

SEQ ID NO: 295 - protein, 25 aa, Artificial Sequence
  Scaffold Protein
GAQESKKKKKKRFSFKKSFKLSGFS

SEQ ID NO: 296 - protein, 24 aa, Artificial Sequence
  Scaffold Protein
GAQESKKKKKKRFSFKKSFKLSGF

SEQ ID NO: 297 - protein, 23 aa, Artificial Sequence
  Scaffold Protein
GAQESKKKKKKRFSFKKSFKLSG

SEQ ID NO: 298 - protein, 22 aa, Artificial Sequence
  Scaffold Protein
GAQESKKKKKKRFSFKKSFKLS

SEQ ID NO: 299 - protein, 21 aa, Artificial Sequence
  Scaffold Protein
GAQESKKKKKKRFSFKKSFKL

SEQ ID NO: 300 - protein, 20 aa, Artificial Sequence
  Scaffold Protein
GAQESKKKKKKRFSFKKSFK

SEQ ID NO: 301 - protein, 19 aa, Artificial Sequence
  Scaffold Protein
GAQESKKKKKKRFSFKKSF

SEQ ID NO: 302 - protein, 18 aa, Artificial Sequence
  Scaffold Protein
GAQESKKKKKKRFSFKKS

SEQ ID NO: 303 - protein, 17 aa, Artificial Sequence
  Scaffold Protein
GAQESKKKKKKRFSFKK

SEQ ID NO: 304 - protein, 16 aa, Artificial Sequence
  Scaffold Protein
GAQESKKKKKKRFSFK

SEQ ID NO: 305 - protein, 15 aa, Artificial Sequence
  Scaffold Protein
GAQESKKKKKKRFSF

SEQ ID NO: 306 - protein, 14 aa, Artificial Sequence
  Scaffold Protein
GAQESKKKKKKRFS

SEQ ID NO: 307 - protein, 13 aa, Artificial Sequence
  Scaffold Protein
GAQESKKKKKKRF

SEQ ID NO: 308 - protein, 12 aa, Artificial Sequence
  Scaffold Protein
GAQESKKKKKKR

SEQ ID NO: 309 - protein, 11 aa, Artificial Sequence
  Scaffold Protein
GAQESKKKKKK

SEQ ID NO: 310 - protein, 10 aa, Artificial Sequence
  Scaffold Protein
GAQESKKKKK

SEQ ID NO: 311 - protein, 9 aa, Artificial Sequence
  Scaffold Protein
GAQESKKKK

SEQ ID NO: 312 - protein, 8 aa, Artificial Sequence
  Scaffold Protein
GAQESKKK

SEQ ID NO: 313 - protein, 7 aa, Artificial Sequence
  Scaffold Protein
GAQESKK

SEQ ID NO: 314 - protein, 30 aa, Artificial Sequence
  Scaffold Protein
GSQSSKKKKKKFSFKKPFKLSGLSFKRNRK

SEQ ID NO: 315 - protein, 29 aa, Artificial Sequence
  Scaffold Protein
GSQSSKKKKKKFSFKKPFKLSGLSFKRNR

SEQ ID NO: 316 - protein, 28 aa, Artificial Sequence
  Scaffold Protein
GSQSSKKKKKKFSFKKPFKLSGLSFKRN

SEQ ID NO: 317 - protein, 27 aa, Artificial Sequence
  Scaffold Protein
GSQSSKKKKKKFSFKKPFKLSGLSFKR

SEQ ID NO: 318 - protein, 26 aa, Artificial Sequence
  Scaffold Protein
GSQSSKKKKKKFSFKKPFKLSGLSFK

SEQ ID NO: 319 - protein, 25 aa, Artificial Sequence
  Scaffold Protein
GSQSSKKKKKKFSFKKPFKLSGLSF

SEQ ID NO: 320 - protein, 24 aa, Artificial Sequence
  Scaffold Protein
GSQSSKKKKKKFSFKKPFKLSGLS

SEQ ID NO: 321 - protein, 23 aa, Artificial Sequence
  Scaffold Protein
GSQSSKKKKKKFSFKKPFKLSGL

SEQ ID NO: 322 - protein, 22 aa, Artificial Sequence
  Scaffold Protein
GSQSSKKKKKKFSFKKPFKLSG

SEQ ID NO: 323 - protein, 21 aa, Artificial Sequence
  Scaffold Protein
GSQSSKKKKKKFSFKKPFKLS

SEQ ID NO: 324 - protein, 20 aa, Artificial Sequence
  Scaffold Protein
GSQSSKKKKKKFSFKKPFKL

SEQ ID NO: 325 - protein, 19 aa, Artificial Sequence
  Scaffold Protein
GSQSSKKKKKKFSFKKPFK

SEQ ID NO: 326 - protein, 18 aa, Artificial Sequence
  Scaffold Protein
GSQSSKKKKKKFSFKKPF

SEQ ID NO: 327 - protein, 17 aa, Artificial Sequence
  Scaffold Protein
GSQSSKKKKKKFSFKKP

SEQ ID NO: 328 - protein, 16 aa, Artificial Sequence
  Scaffold Protein
GSQSSKKKKKKFSFKK

SEQ ID NO: 329 - protein, 15 aa, Artificial Sequence
  Scaffold Protein
GSQSSKKKKKKFSFK

SEQ ID NO: 330 - protein, 14 aa, Artificial Sequence
  Scaffold Protein
GSQSSKKKKKKFSF

SEQ ID NO: 331 - protein, 13 aa, Artificial Sequence
  Scaffold Protein
GSQSSKKKKKKFS

SEQ ID NO: 332 - protein, 12 aa, Artificial Sequence
  Scaffold Protein
GSQSSKKKKKKF

SEQ ID NO: 333 - protein, 11 aa, Artificial Sequence
  Scaffold Protein
GSQSSKKKKKK

SEQ ID NO: 334 - protein, 10 aa, Artificial Sequence
  Scaffold Protein
GSQSSKKKKK

SEQ ID NO: 335 - protein, 9 aa, Artificial Sequence
  Scaffold Protein
GSQSSKKKK

SEQ ID NO: 336 - protein, 8 aa, Artificial Sequence
  Scaffold Protein
GSQSSKKK

SEQ ID NO: 337 - protein, 7 aa, Artificial Sequence
  Scaffold Protein
GSQSSKK

SEQ ID NO: 338 - protein, 7 aa, Artificial Sequence
  fusion protein
GGKFSKK

SEQ ID NO: 339 - protein, 7 aa, Artificial Sequence
  fusion protein
GGKFAKK

SEQ ID NO: 340 - protein, 7 aa, Artificial Sequence
  fusion protein
GGKSSKK

SEQ ID NO: 341 - protein, 7 aa, Artificial Sequence
  fusion protein
GGKSAKK

SEQ ID NO: 342 - protein, 7 aa, Artificial Sequence
  fusion protein
GGKQAKK

SEQ ID NO: 343 - protein, 7 aa, Artificial Sequence
  fusion protein
GGQLSKK

SEQ ID NO: 344 - protein, 7 aa, Artificial Sequence
  fusion protein
GGQLAKK

SEQ ID NO: 345 - protein, 7 aa, Artificial Sequence
  fusion protein
GGQFSKK

SEQ ID NO: 346 - protein, 7 aa, Artificial Sequence
  fusion protein
GGQFAKK

SEQ ID NO: 347 - protein, 7 aa, Artificial Sequence
  fusion protein
GGQSSKK

SEQ ID NO: 348 - protein, 7 aa, Artificial Sequence
  fusion protein
GGQSAKK

SEQ ID NO: 349 - protein, 7 aa, Artificial Sequence
  fusion protein
GGQQSKK

SEQ ID NO: 350 - protein, 7 aa, Artificial Sequence
  fusion protein
GGQQAKK

SEQ ID NO: 351 - protein, 7 aa, Artificial Sequence
  fusion protein
GAKLAKK

SEQ ID NO: 352 - protein, 7 aa, Artificial Sequence
  fusion protein
GAKFSKK

SEQ ID NO: 353 - protein, 7 aa, Artificial Sequence
  fusion protein
GAKFAKK

SEQ ID NO: 354 - protein, 7 aa, Artificial Sequence
  fusion protein
GAKSSKK

SEQ ID NO: 355 - protein, 7 aa, Artificial Sequence
  fusion protein
GAKSAKK

SEQ ID NO: 356 - protein, 7 aa, Artificial Sequence
  fusion protein
GAKQSKK

SEQ ID NO: 357 - protein, 7 aa, Artificial Sequence
  fusion protein
GAKQAKK

SEQ ID NO: 358 - protein, 7 aa, Artificial Sequence
  fusion protein
GAQLSKK

SEQ ID NO: 359 - protein, 7 aa, Artificial Sequence
  fusion protein
GAQLAKK

SEQ ID NO: 360 - protein, 7 aa, Artificial Sequence
  fusion protein
GAQFSKK

SEQ ID NO: 361 - protein, 7 aa, Artificial Sequence
  fusion protein
GAQFAKK

SEQ ID NO: 362 - protein, 7 aa, Artificial Sequence
  fusion protein
GAQSSKK

SEQ ID NO: 363 - protein, 7 aa, Artificial Sequence
  fusion protein
GAQSAKK

SEQ ID NO: 364 - protein, 7 aa, Artificial Sequence
  fusion protein
GAQQSKK

SEQ ID NO: 365 - protein, 7 aa, Artificial Sequence
  fusion protein
GAQQAKK

SEQ ID NO: 366 - protein, 7 aa, Artificial Sequence
  fusion protein
GSKLSKK

SEQ ID NO: 367 - protein, 7 aa, Artificial Sequence
  fusion protein
GSKLAKK

SEQ ID NO: 368 - protein, 7 aa, Artificial Sequence
  fusion protein
GSKFSKK

SEQ ID NO: 369 - protein, 7 aa, Artificial Sequence
  fusion protein
GSKFAKK

SEQ ID NO: 370 - protein, 7 aa, Artificial Sequence
  fusion protein
GSKSSKK

SEQ ID NO: 371 - protein, 7 aa, Artificial Sequence
  fusion protein
GSKSAKK

SEQ ID NO: 372 - protein, 7 aa, Artificial Sequence
  fusion protein
GSKQSKK

SEQ ID NO: 373 - protein, 7 aa, Artificial Sequence
  fusion protein
GSKQAKK

SEQ ID NO: 374 - protein, 7 aa, Artificial Sequence
  fusion protein
GSQLSKK

SEQ ID NO: 375 - protein, 7 aa, Artificial Sequence
  fusion protein
GSQLAKK

SEQ ID NO: 376 - protein, 7 aa, Artificial Sequence
  fusion protein
GSQFSKK

SEQ ID NO: 377 - protein, 7 aa, Artificial Sequence
  fusion protein
GSQFAKK

SEQ ID NO: 378 - protein, 7 aa, Artificial Sequence
  fusion protein
GSQSAKK

SEQ ID NO: 379 - protein, 7 aa, Artificial Sequence
  fusion protein
GSQQSKK

SEQ ID NO: 380 - protein, 7 aa, Artificial Sequence
  fusion protein
GSQQAKK

SEQ ID NO: 381 - protein, 6 aa, Artificial Sequence
  fusion protein
GGKFSK

SEQ ID NO: 382 - protein, 6 aa, Artificial Sequence
  fusion protein
GGKFAK

SEQ ID NO: 383 - protein, 6 aa, Artificial Sequence
  fusion protein
GGKSSK

SEQ ID NO: 384 - protein, 6 aa, Artificial Sequence
  fusion protein
GGKSAK

SEQ ID NO: 385 - protein, 6 aa, Artificial Sequence
  fusion protein
GGKQAK

SEQ ID NO: 386 - protein, 6 aa, Artificial Sequence
  fusion protein
GGQLSK

SEQ ID NO: 387 - protein, 6 aa, Artificial Sequence
  fusion protein
GGQLAK

SEQ ID NO: 388 - protein, 6 aa, Artificial Sequence
  fusion protein
GGQFSK

SEQ ID NO: 389 - protein, 6 aa, Artificial Sequence
  fusion protein
GGQFAK

SEQ ID NO: 390 - protein, 6 aa, Artificial Sequence
  fusion protein
GGQSSK

SEQ ID NO: 391 - protein, 6 aa, Artificial Sequence
  fusion protein
GGQSAK

SEQ ID NO: 392 - protein, 6 aa, Artificial Sequence
  fusion protein
GGQQSK

SEQ ID NO: 393 - protein, 6 aa, Artificial Sequence
  fusion protein
GGQQAK

SEQ ID NO: 394 - protein, 6 aa, Artificial Sequence
  fusion protein
GAKLAK

SEQ ID NO: 395 - protein, 6 aa, Artificial Sequence
  fusion protein
GAKFSK

SEQ ID NO: 396 - protein, 6 aa, Artificial Sequence
  fusion protein
GAKFAK

SEQ ID NO: 397 - protein, 6 aa, Artificial Sequence
  fusion protein
GAKSSK

SEQ ID NO: 398 - protein, 6 aa, Artificial Sequence
  fusion protein
GAKSAK

SEQ ID NO: 399 - protein, 6 aa, Artificial Sequence
  fusion protein
GAKQSK

SEQ ID NO: 400 - protein, 6 aa, Artificial Sequence
  fusion protein
GAKQAK

SEQ ID NO: 401 - protein, 6 aa, Artificial Sequence
  fusion protein
GAQLSK

SEQ ID NO: 402 - protein, 6 aa, Artificial Sequence
  fusion protein
GAQLAK

SEQ ID NO: 403 - protein, 6 aa, Artificial Sequence
  fusion protein
GAQFSK

SEQ ID NO: 404 - protein, 6 aa, Artificial Sequence
  fusion protein
GAQFAK

SEQ ID NO: 405 - protein, 6 aa, Artificial Sequence
  fusion protein
GAQSSK

SEQ ID NO: 406 - protein, 6 aa, Artificial Sequence
  fusion protein
GAQSAK

SEQ ID NO: 407 - protein, 6 aa, Artificial Sequence
  fusion protein
GAQQSK

SEQ ID NO: 408 - protein, 6 aa, Artificial Sequence
  fusion protein
GAQQAK

SEQ ID NO: 409 - protein, 6 aa, Artificial Sequence
  fusion protein
GSKLSK

SEQ ID NO: 410 - protein, 6 aa, Artificial Sequence
  fusion protein
GSKLAK

SEQ ID NO: 411 - protein, 6 aa, Artificial Sequence
  fusion protein
GSKFSK

SEQ ID NO: 412 - protein, 6 aa, Artificial Sequence
  fusion protein
GSKFAK

SEQ ID NO: 413 - protein, 6 aa, Artificial Sequence
  fusion protein
GSKSSK

SEQ ID NO: 414 - protein, 6 aa, Artificial Sequence
  fusion protein
GSKSAK

SEQ ID NO: 415 - protein, 6 aa, Artificial Sequence
  fusion protein
GSKQSK

SEQ ID NO: 416 - protein, 6 aa, Artificial Sequence
  fusion protein
GSKQAK

SEQ ID NO: 417 - protein, 6 aa, Artificial Sequence
  fusion protein
GSQLSK

SEQ ID NO: 418 - protein, 6 aa, Artificial Sequence
  fusion protein
GSQLAK

SEQ ID NO: 419 - protein, 6 aa, Artificial Sequence
  fusion protein
GSQFSK

SEQ ID NO: 420 - protein, 6 aa, Artificial Sequence
  fusion protein
GSQFAK

SEQ ID NO: 421 - protein, 6 aa, Artificial Sequence
  fusion protein
GSQSSK

SEQ ID NO: 422 - protein, 6 aa, Artificial Sequence
  fusion protein
GSQSAK

SEQ ID NO: 423 - protein, 6 aa, Artificial Sequence
  fusion protein
GSQQSK

SEQ ID NO: 424 - protein, 6 aa, Artificial Sequence
  fusion protein
GSQQAK

SEQ ID NO: 425 - protein, 8 aa, Artificial Sequence
  Fusion Protein
  misc_feature (2)..(2): Xaa can be any naturally occurring amino acid
GXKLSKKK